European Patent Application EP 4 269 447 A1, published November 1, 2023. Title: COMPLEX OF ANTI-IL-4R ANTIBODY OR ANTIGEN-BINDING FRAGMENT THEREOF AND MEDICAL USE THEREOF. Applicant: Jiangsu Hengrui Pharmaceuticals Co., Ltd. Shanghai Shengdi Pharmaceutical Co., Ltd. Application PCT/CN2021/140310. The sequence listing filed with the application follows.

SEQUENCE LISTING (67 sequences)

SEQ ID NO: 1 - protein, 118 aa, Mus musculus
EVQLVESGGGLVKPGGSLKLSCAASGFTFSDYGMHWVRQAPEKGLEWVAFISSGSSIIYYADIVKGRSTISRDNAKNTLFLQMTSLRSEDTAMYYCTRGNKRGFFDYWGQGTILTVSS

SEQ ID NO: 2 - protein, 108 aa, Mus musculus
QIVLTQSPALMSASPGEKVTMTCNASSSVSYMYWYQRKPRSSPKPWIYLTSNLASGVPVRFSGSGSGTSYSLTISSMEAEDAATYYCQQWRSNPPMLTFGSGTKLEVK

SEQ ID NO: 3 - protein, 10 aa, Mus musculus
GFTFSDYGMH

SEQ ID NO: 4 - protein, 17 aa, Mus musculus
FISSGSSIIYYADIVKG

SEQ ID NO: 5 - protein, 9 aa, Mus musculus
GNKRGFFDY

SEQ ID NO: 6 - protein, 10 aa, Mus musculus
NASSSVSYMY

SEQ ID NO: 7 - protein, 7 aa, Mus musculus
LTSNLAS

SEQ ID NO: 8 - protein, 11 aa, Mus musculus
QQWRSNPPMLT

SEQ ID NO: 9 - protein, 125 aa, Mus musculus
QVQLQQPGTELLKPGASVSLSCKASGYTFTSYWMHWVKQRPGQGLEWIGLIHPNSDTTKFSENFKTRATLTIDKSSSTAYMKLSSLTSEDSAVYYCAKSKIITTIVARHWYFDVWGTGTTVTVSS

SEQ ID NO: 10 - protein, 111 aa, Mus musculus
DIVLTQSPPSLAVSLGQRATISCKASQSVDYGGDSYMNWYQQKLGQPPKVLIYAASNLESGIPARFSGSGSGTDFTLNIHPVEEEDVATYYCQHSNENPPTFGGGTKLEIK

SEQ ID NO: 11 - protein, 10 aa, Mus musculus
GYTFTSYWMH

SEQ ID NO: 12 - protein, 17 aa, Mus musculus
LIHPNSDTTKFSENFKT

SEQ ID NO: 13 - protein, 16 aa, Mus musculus
SKIITTIVARHWYFDV

SEQ ID NO: 14 - protein, 15 aa, Mus musculus
KASQSVDYGGDSYMN

SEQ ID NO: 15 - protein, 7 aa, Mus musculus
AASNLES

SEQ ID NO: 16 - protein, 9 aa, Mus musculus
QHSNENPPT

SEQ ID NO: 17 - protein, 445 aa, Artificial Sequence
  Synthesized sequence (hu25G7 HC)
EVQLVESGGGLVQPGGSLRLSCAASGFTFSDYGMHWVRQAPGKGLEWVAFISSGSSIIYYADIVKGRSTISRDNAKNSLYLQMNSLRAEDTAVYYCTRGNKRGFFDYWGQGTLVTVSSASTKGPSVFPLAPCSRSTSESTAALGCLVKDYFPEPVTVSWNSGALTSGVHTFPAVLQSSGLYSLSSVVTVPSSSLGTKTYTCNVDHKPSNTKVDKRVESKYGPPCPPCPAPEFLGGPSVFLFPPKPKDTLMISRTPEVTCVVVDVSQEDPEVQFNWYVDGVEVHNAKTKPREEQFNSTYRVVSVLTVLHQDWLNGKEYKCKVSNKGLPSSIEKTISKAKGQPREPQVYTLPPSQEEMTKNQVSLTCLVKGFYPSDIAVEWESNGQPENNYKTTPPVLDSDGSFFLYSRLTVDKSRWQEGNVFSCSVMHEALHNHYTQKSLSLSLGK

SEQ ID NO: 18 - protein, 215 aa, Artificial Sequence
  Synthesized squence (hu25G7 LC)
EIVLTQSPATLSLSPGERATLSCNASSSVSYMYWYQQKPGQAPRLLIYLTSNLASGIPARFSGSGSGTDFTLTISSLEPEDFAVYYCQQWRSNPPMLTFGGGTKVEIKRTVAAPSVFIFPPSDEQLKSGTASVVCLLNNFYPREAKVQWKVDNALQSGNSQESVTEQDSKDSTYSLSSTLTLSKADYEKHKVYACEVTHQGLSSPVTKSFNRGEC

SEQ ID NO: 19 - protein, 455 aa, Artificial Sequence
  Synthesized sequence (hu7B10 HC)
EVQLVQSGAEVKKPGASVKVSCKASGYTFTSYWMHWVRQAPGQGLEWMGLIHPNSDTTKFSENFKTRVTMTIDTSISTAYMELSRLRSDDTAVYYCAKSKIITTIVARHWYFDVWGQGTTVTVSSASTKGPSVFPLAPSSKSTSGGTAALGCLVKDYFPEPVTVSWNSGALTSGVHTFPAVLQSSGLYSLSSVVTVPSSSLGTQTYICNVNHKPSNTKVDKKVEPKSCDKTHTCPPCPAPELLGGPSVFLFPPKPKDTLMISRTPEVTCVVVDVSHEDPEVKFNWYVDGVEVHNAKTKPREEQYNSTYRVVSVLTVLHQDWLNGKEYKCKVSNKALPAPIEKTISKAKGQPREPQVYTLPPSREEMTKNQVSLTCLVKGFYPSDIAVEWESNGQPENNYKTTPPVLDSDGSFFLYSKLTVDKSRWQQGNVFSCSVMHEALHNHYTQKSLSLSPGK

SEQ ID NO: 20 - protein, 218 aa, Artificial Sequence
  Synthesized sequence (hu7B10 LC)
DIVLTQTPLSLSVTPGQPASISCKASQSVDYGGDSYMNWYLQKPGQPPQLLIYAASNLESGVPDRFSGSGSGTDFTLKISRVEAEDVGVYYCQHSNENPPTFGGGTKVEIKRTVAAPSVFIFPPSDEQLKSGTASVVCLLNNFYPREAKVQWKVDNALQSGNSQESVTEQDSKDSTYSLSSTLTLSKADYEKHKVYACEVTHQGLSSPVTKSFNRGEC

SEQ ID NO: 21 - protein, 98 aa, Homo sapiens
EVQLVESGGGLVQPGGSLRLSCAASGFTFSSYSMNWVRQAPGKGLEWVSYISSSSSTIYYADSVKGRFTISRDNAKNSLYLQMNSLRAEDTAVYYCAR

SEQ ID NO: 22 - protein, 95 aa, Homo sapiens
EIVLTQSPATLSLSPGERATLSCRASQSVSSYLAWYQQKPGQAPRLLIYDASNRATGIPARFSGSGSGTDFTLTISSLEPEDFAVYYCQQRSNWP

SEQ ID NO: 23 - protein, 98 aa, Homo sapiens
QVQLVQSGAEVKKPGASVKVSCKASGYTFTGYYMHWVRQAPGQGLEWMGWINPNSGGTNYAQKFQGRVTMTRDTSISTAYMELSRLRSDDTAVYYCAR

SEQ ID NO: 24 - protein, 100 aa, Homo sapiens
DIVMTQTPLSLSVTPGQPASISCKSSQSLLHSDGKTYLYWYLQKPGQPPQLLIYEVSNRFSGVPDRFSGSGSGTDFTLKISRVEAEDVGVYYCMQSIQLP

SEQ ID NO: 25 - protein, 118 aa, Artificial Sequence
  Synthesized sequence (hu25G7-VH-a)
EVQLVESGGGLVQPGGSLRLSCAASGFTFSDYGMHWVRQAPGKGLEWVAFISSGSSIIYYADIVKGRFTISRDNAKNSLYLQMNSLRAEDTAVYYCARGNKRGFFDYWGQGTLVTVSS

SEQ ID NO: 26 - protein, 118 aa, Artificial Sequence
  Synthesized sequence (hu25G7-VH-b)
EVQLVESGGGLVQPGGSLRLSCAASGFTFSDYGMHWVRQAPGKGLEWVAFISSGSSIIYYADIVKGRFTISRDNAKNSLYLQMNSLRAEDTAVYYCTRGNKRGFFDYWGQGTLVTVSS

SEQ ID NO: 27 - protein, 118 aa, Artificial Sequence
  Synthesized sequence (hu25G7-VH-c)
EVQLVESGGGLVQPGGSLRLSCAASGFTFSDYGMHWVRQAPGKGLEWVAFISSGSSIIYYADIVKGRSTISRDNAKNSLYLQMNSLRAEDTAVYYCTRGNKRGFFDYWGQGTLVTVSS

SEQ ID NO: 28 - protein, 108 aa, Artificial Sequence
  Synthesized sequence (hu25G7-VL-a)
EIVLTQSPATLSLSPGERATLSCNASSSVSYMYWYQQKPGQAPRLLIYLTSNLASGIPARFSGSGSGTDFTLTISSLEPEDFAVYYCQQWRSNPPMLTFGGGTKVEIK

SEQ ID NO: 29 - protein, 108 aa, Artificial Sequence
  Synthesized sequence (hu25G7-VL-b)
EIVLTQSPATLSLSPGERATLSCNASSSVSYMYWYQQKPGQAPRLLIYLTSNLASGIPARFSGSGSGTDYTLTISSLEPEDFAVYYCQQWRSNPPMLTFGGGTKVEIK

SEQ ID NO: 30 - protein, 108 aa, Artificial Sequence
  Synthesized sequence (hu25G7-VL-c)
EIVLTQSPATLSLSPGERATLSCNASSSVSYMYWYQQKPGQAPRPWIYLTSNLASGIPARFSGSGSGTDYTLTISSLEPEDFAVYYCQQWRSNPPMLTFGGGTKVEIK

SEQ ID NO: 31 - protein, 125 aa, Artificial Sequence
  Synthesized sequence (hu7B10-VH-a)
EVQLVQSGAEVKKPGASVKVSCKASGYTFTSYWMHWVRQAPGQGLEWMGLIHPNSDTTKFSENFKTRVTMTRDTSISTAYMELSRLRSDDTAVYYCARSKIITTIVARHWYFDVWGQGTTVTVSS

SEQ ID NO: 32 - protein, 125 aa, Artificial Sequence
  Synthesized sequence (hu7B10-VH-b)
EVQLVQSGAEVKKPGASVKVSCKASGYTFTSYWMHWVRQAPGQGLEWMGLIHPNSDTTKFSENFKTRVTMTIDTSISTAYMELSRLRSDDTAVYYCAKSKIITTIVARHWYFDVWGQGTTVTVSS

SEQ ID NO: 33 - protein, 125 aa, Artificial Sequence
  Synthesized sequence (hu7B10-VH-c)
EVQLVQSGAEVKKPGASVKVSCKASGYTFTSYWMHWVRQAPGQGLEWMGLIHPNSDTTKFSENFKTRVTLTIDKSISTAYMELSRLRSDDTAVYYCAKSKIITTIVARHWYFDVWGQGTTVTVSS

SEQ ID NO: 34 - protein, 111 aa, Artificial Sequence
  Synthesized sequence (hu7B10-VL-a)
DIVMTQTPLSLSVTPGQPASISCKASQSVDYGGDSYMNWYLQKPGQPPQLLIYAASNLESGVPDRFSGSGSGTDFTLKISRVEAEDVGVYYCQHSNENPPTFGGGTKVEIK

SEQ ID NO: 35 - protein, 111 aa, Artificial Sequence
  Synthesized sequence (hu7B10-VL-b)
DIVLTQTPLSLSVTPGQPASISCKASQSVDYGGDSYMNWYLQKPGQPPQLLIYAASNLESGVPDRFSGSGSGTDFTLKISRVEAEDVGVYYCQHSNENPPTFGGGTKVEIK

SEQ ID NO: 36 - protein, 111 aa, Artificial Sequence
  Synthesized sequence (hu7B10-VL-c)
DIVMTQTPLSLSVTPGQPASISCKASQSVDYGGDSYMNWYLQKPGQPPQLLIYAASNLESGIPDRFSGSGSGTDFTLKISRVEAEDVGVYYCQHSNENPPTFGGGTKVEIK

SEQ ID NO: 37 - protein, 108 aa, Artificial Sequence
  Synthesized sequence (hu25G7-A LCVR)
EIVLTQSPATLSLSPGERATLSCRASSSVPYMYWYQQKPGQAPRLLIYLTSNLASGIPARFSGSGSGTDFTLTISSLEPEDFAVYYCQQWRAYPPMLTFGGGTKVEIK

SEQ ID NO: 38 - protein, 10 aa, Artificial Sequence
  Synthesized sequence (LCDR1)
RASSSVPYMY

SEQ ID NO: 39 - protein, 7 aa, Artificial Sequence
  Synthesized sequence (LCDR2)
LASSRPS

SEQ ID NO: 40 - protein, 11 aa, Artificial Sequence
  Synthesized sequence (LCDR3)
QQWRAYPPMLT

SEQ ID NO: 41 - protein, 108 aa, Artificial Sequence
  Synthesized sequence (hu25G7-B LCVR)
EIVLTQSPATLSLSPGERATLSCRASPGVPPLAWYQQKPGQAPRLLIYLASSRPSGIPARFSGSGSGTDFTLTISSLEPEDFAVYYCQQWRSNPPMLTFGGGTKVEIK

SEQ ID NO: 42 - protein, 10 aa, Artificial Sequence
  Synthesized sequence (LCDR1)
RASPGVPPLA

SEQ ID NO: 43 - protein, 118 aa, Artificial Sequence
  Synthesized sequence (hu25G7-VH)
EVQLVESGGGLVQPGGSLRLSCAASGFTFSDYGMHWVRQAPGKGLEWVAFISSGSSIIYYADIVKGRSTISRDNAKNTLYLQMNSLRAEDTAVYYCTRGNKRGFFDYWGQGTLVTVSS

SEQ ID NO: 44 - protein, 445 aa, Artificial Sequence
  Synthesized sequence (hu25G7 HC)
EVQLVESGGGLVQPGGSLRLSCAASGFTFSDYGMHWVRQAPGKGLEWVAFISSGSSIIYYADIVKGRSTISRDNAKNTLYLQMNSLRAEDTAVYYCTRGNKRGFFDYWGQGTLVTVSSASTKGPSVFPLAPCSRSTSESTAALGCLVKDYFPEPVTVSWNSGALTSGVHTFPAVLQSSGLYSLSSVVTVPSSSLGTKTYTCNVDHKPSNTKVDKRVESKYGPPCPPCPAPEFLGGPSVFLFPPKPKDTLMISRTPEVTCVVVDVSQEDPEVQFNWYVDGVEVHNAKTKPREEQFNSTYRVVSVLTVLHQDWLNGKEYKCKVSNKGLPSSIEKTISKAKGQPREPQVYTLPPSQEEMTKNQVSLTCLVKGFYPSDIAVEWESNGQPENNYKTTPPVLDSDGSFFLYSRLTVDKSRWQEGNVFSCSVMHEALHNHYTQKSLSLSLGK

SEQ ID NO: 45 - protein, 215 aa, Artificial Sequence
  Synthesized sequence (hu25G7-A LC)
EIVLTQSPATLSLSPGERATLSCRASSSVPYMYWYQQKPGQAPRLLIYLTSNLASGIPARFSGSGSGTDFTLTISSLEPEDFAVYYCQQWRAYPPMLTFGGGTKVEIKRTVAAPSVFIFPPSDEQLKSGTASVVCLLNNFYPREAKVQWKVDNALQSGNSQESVTEQDSKDSTYSLSSTLTLSKADYEKHKVYACEVTHQGLSSPVTKSFNRGEC

SEQ ID NO: 46 - protein, 215 aa, Artificial Sequence
  Synthesized sequence (hu25G7-B LC)
EIVLTQSPATLSLSPGERATLSCRASPGVPPLAWYQQKPGQAPRLLIYLASSRPSGIPARFSGSGSGTDFTLTISSLEPEDFAVYYCQQWRSNPPMLTFGGGTKVEIKRTVAAPSVFIFPPSDEQLKSGTASVVCLLNNFYPREAKVQWKVDNALQSGNSQESVTEQDSKDSTYSLSSTLTLSKADYEKHKVYACEVTHQGLSSPVTKSFNRGEC

SEQ ID NO: 47 - protein, 118 aa, Artificial Sequence
  Synthesized sequence (hu25G7-VH-44)
EVQLVESGGGLVQPGGSLRLSCAASGFTFSDYGMHWVRQAPGKCLEWVAFISSGSSIIYYADIVKGRSTISRDNAKNTLYLQMNSLRAEDTAVYYCTRGNKRGFFDYWGQGTLVTVSS

SEQ ID NO: 48 - protein, 108 aa, Artificial Sequence
  Synthesized sequence (hu25G7-VL-100)
EIVLTQSPATLSLSPGERATLSCRASSSVPYMYWYQQKPGQAPRLLIYLTSNLASGIPARFSGSGSGTDFTLTISSLEPEDFAVYYCQQWRAYPPMLTFGCGTKVEIK

SEQ ID NO: 49 - protein, 345 aa, Artificial Sequence
  Synthesized sequence (PE38KDEL)
EGGSLAALTAHQACHLPLETFTRHRQPRGWEQLEQCGYPVQRLVALYLAARLSWNQVDQVIRNALASPGSGGDLGEAIREQPEQARLALTLAAAESERFVRQGTGNDEAGAANGPADSGDALLERNYPTGAEFLGDGGDVSFSTRGTQNWTVERLLQAHRQLEERGYVFVGYHGTFLEAAQSIVFGGVRARSQDLDAIWRGFYIAGDPALAYGYAQDQEPDARGRIRNGALLRVYVPRSSLPGFYRTSLTLAAPEAAGEVERLIGHPLPLRLDAITGPEEEGGRLETILGWPLAERTVVIPSAIPTDPRNVGGDLDPSSIPDKEQAISALPDYASQPGKPPKDEL

SEQ ID NO: 50 - protein, 6 aa, Artificial Sequence
  Synthesized sequence (linker1)
ASGGPE

SEQ ID NO: 51 - protein, 15 aa, Artificial Sequence
  Synthesized sequence (Linker 2)
GGGGSGGGGSGGGGS

SEQ ID NO: 52 - protein, 592 aa, Artificial Sequence
  Synthesized sequence (25G7-(scdsFv)-PE38KDEL)
EVQLVESGGGLVQPGGSLRLSCAASGFTFSDYGMHWVRQAPGKCLEWVAFISSGSSIIYYADIVKGRSTISRDNAKNTLYLQMNSLRAEDTAVYYCTRGNKRGFFDYWGQGTLVTVSSGGGGSGGGGSGGGGSEIVLTQSPATLSLSPGERATLSCRASSSVPYMYWYQQKPGQAPRLLIYLTSNLASGIPARFSGSGSGTDFTLTISSLEPEDFAVYYCQQWRAYPPMLTFGCGTKVEIKASGGPEEGGSLAALTAHQACHLPLETFTRHRQPRGWEQLEQCGYPVQRLVALYLAARLSWNQVDQVIRNALASPGSGGDLGEAIREQPEQARLALTLAAAESERFVRQGTGNDEAGAANGPADSGDALLERNYPTGAEFLGDGGDVSFSTRGTQNWTVERLLQAHRQLEERGYVFVGYHGTFLEAAQSIVFGGVRARSQDLDAIWRGFYIAGDPALAYGYAQDQEPDARGRIRNGALLRVYVPRSSLPGFYRTSLTLAAPEAAGEVERLIGHPLPLRLDAITGPEEEGGRLETILGWPLAERTVVIPSAIPTDPRNVGGDLDPSSIPDKEQAISALPDYASQPGKPPKDEL

SEQ ID NO: 53 - protein, 592 aa, Artificial Sequence
  Synthesized sequence (25G7-(scFv)-PE38KDEL)
EVQLVESGGGLVQPGGSLRLSCAASGFTFSDYGMHWVRQAPGKGLEWVAFISSGSSIIYYADIVKGRSTISRDNAKNTLYLQMNSLRAEDTAVYYCTRGNKRGFFDYWGQGTLVTVSSGGGGSGGGGSGGGGSEIVLTQSPATLSLSPGERATLSCRASSSVPYMYWYQQKPGQAPRLLIYLTSNLASGIPARFSGSGSGTDFTLTISSLEPEDFAVYYCQQWRAYPPMLTFGGGTKVEIKASGGPEEGGSLAALTAHQACHLPLETFTRHRQPRGWEQLEQCGYPVQRLVALYLAARLSWNQVDQVIRNALASPGSGGDLGEAIREQPEQARLALTLAAAESERFVRQGTGNDEAGAANGPADSGDALLERNYPTGAEFLGDGGDVSFSTRGTQNWTVERLLQAHRQLEERGYVFVGYHGTFLEAAQSIVFGGVRARSQDLDAIWRGFYIAGDPALAYGYAQDQEPDARGRIRNGALLRVYVPRSSLPGFYRTSLTLAAPEAAGEVERLIGHPLPLRLDAITGPEEEGGRLETILGWPLAERTVVIPSAIPTDPRNVGGDLDPSSIPDKEQAISALPDYASQPGKPPKDEL

SEQ ID NO: 54 - protein, 12 aa, Artificial Sequence
  Synthesized sequence (linker)
GKSSGSGSESKS

SEQ ID NO: 55 - protein, 14 aa, Artificial Sequence
  Synthesized sequence (linker)
EGKSSGSGSESKEF

SEQ ID NO: 56 - protein, 14 aa, Artificial Sequence
  Synthesized sequence (linker)
GSTSGSGKSSEGKG

SEQ ID NO: 57 - protein, 18 aa, Artificial Sequence
  Synthesized sequence (linker)
GSTSGSGKSSEGSGSTKG

SEQ ID NO: 58 - protein, 18 aa, Artificial Sequence
  Synthesized sequence (linker)
GSTSGSGKPGSGEGSTKG

SEQ ID NO: 59 - protein, 5 aa, Artificial Sequence
  Synthesized sequence (linker)
SRSSG

SEQ ID NO: 60 - protein, 5 aa, Artificial Sequence
  Synthesized sequence (linker)
SGSSC

SEQ ID NO: 61 - protein, 5 aa, Artificial Sequence
  Synthesized sequence (linker)
GGGGS

SEQ ID NO: 62 - protein, 7 aa, Artificial Sequence
  Synthesized sequence (linker)
ASGCGPE

SEQ ID NO: 63 - protein, 8 aa, Artificial Sequence
  Synthesized sequence (linker)
ASGCCGPE

SEQ ID NO: 64 - protein, 9 aa, Artificial Sequence
  Synthesized sequence (linker)
ASGCGSCPE

SEQ ID NO: 65 - protein, 10 aa, Artificial Sequence
  Synthesized sequence (linker)
ASCGTTGCPE

SEQ ID NO: 66 - protein, 14 aa, Artificial Sequence
  Synthesized sequence (linker)
KASGKKYGCKKGPE

SEQ ID NO: 67 - protein, 10 aa, Artificial Sequence
  Synthesized sequence (linker)
KGGGCAGGPE